European Patent Application EP 4 628 512 A1, published October 8, 2025. Title: Trispecific fusion proteins and uses thereof. Applicant: 信达生物制药(苏州)有限公司. The sequence listing filed with the application follows.

SEQUENCE LISTING (70 sequences)

SEQ ID NO: 1 - protein, 10 aa, synthetic construct
GSSFSPYAMG

SEQ ID NO: 2 - protein, 16 aa, synthetic construct
ATSEGGFTLYADSVKG

SEQ ID NO: 3 - protein, 10 aa, synthetic construct
HWRGSDPENY

SEQ ID NO: 4 - protein, 118 aa, synthetic construct
EVQLVESGGGLVQPGGSLRLSCAASGSSFSPYAMGWYRQAPGKQRELVSATSEGGFTLYADSVKGRFTISRDNSKNTVYLQMNSLRAEDTAVYYCYMHWRGSDPENYWGQGTQVTVSS

SEQ ID NO: 5 - protein, 10 aa, synthetic construct
GFALDYYAIG

SEQ ID NO: 6 - protein, 17 aa, synthetic construct
CISSGEGSTYYADSVKG

SEQ ID NO: 7 - protein, 19 aa, synthetic construct
DSRGDDVACEGLRRNEYDY

SEQ ID NO: 8 - protein, 128 aa, synthetic construct
EVQLLESGGGLVQPGGSLRLSCAASGFALDYYAIGWFRQAPGKGLEGVSCISSGEGSTYYADSVKGRFTISRDNSKNTVYLQMNSLRAEDTAVYYCATDSRGDDVACEGLRRNEYDYWGQGTLVTVSS

SEQ ID NO: 9 - protein, 205 aa, synthetic construct
SDTGRPFVEMYSEIPEIIHMTEGRELVIPCRVTSPNITVTLKKFPLDTLIPDGKRIIWDSRKGFIISNATYKEIGLLTCEATVNGHLYKTNYLTHRQTNTIIDVVLSPSHGIELSVGEKLVLNCTARTELNVGIDFNWEYPSSKHQHKKLVNRDLKTQSGSEMKKFLSTLTIDGVTRSDQGLYTCAASSGLMTKKNSTFVRVHEK

SEQ ID NO: 10 - protein, 10 aa, synthetic construct
GGGGGGGGGG

SEQ ID NO: 11 - protein, 10 aa, synthetic construct
GRPGSGRPGS

SEQ ID NO: 12 - protein, 14 aa, synthetic construct
ESKYGPPCPPCPPC

SEQ ID NO: 13 - protein, 12 aa, synthetic construct
EKTHTCPPCPPC

SEQ ID NO: 14 - protein, 15 aa, synthetic construct
EPKSSPPCPPCPAPC

SEQ ID NO: 15 - protein, 12 aa, synthetic construct
DTTHTCPPCPPC

SEQ ID NO: 16 - protein, 12 aa, synthetic construct
DKTHTCPPCPPC

SEQ ID NO: 17 - protein, 15 aa, synthetic construct
EPKSCDTPPPCPPCP

SEQ ID NO: 18 - protein, 17 aa, synthetic construct
EPKSSDTPPPCPPCPPC

SEQ ID NO: 19 - protein, 16 aa, synthetic construct
DKTHTCPPCPAPELLG

SEQ ID NO: 20 - protein, 24 aa, synthetic construct
ESKYGPPCPPCPPCGGGGGGGGGG

SEQ ID NO: 21 - protein, 22 aa, synthetic construct
EKTHTCPPCPPCGGGGGGGGGG

SEQ ID NO: 22 - protein, 697 aa, synthetic construct
EVQLLESGGGLVQPGGSLRLSCAASGFALDYYAIGWFRQAPGKGLEGVSCISSGEGSTYYADSVKGRFTISRDNSKNTVYLQMNSLRAEDTAVYYCATDSRGDDVACEGLRRNEYDYWGQGTLVTVSSGRPGSGRPGSSDTGRPFVEMYSEIPEIIHMTEGRELVIPCRVTSPNITVTLKKFPLDTLIPDGKRIIWDSRKGFIISNATYKEIGLLTCEATVNGHLYKTNYLTHRQTNTIIDVVLSPSHGIELSVGEKLVLNCTARTELNVGIDFNWEYPSSKHQHKKLVNRDLKTQSGSEMKKFLSTLTIDGVTRSDQGLYTCAASSGLMTKKNSTFVRVHEKDKTHTCPPCPAPELLGGPSVFLFPPKPKDTLMISRTPEVTCVVVDVSHEDPEVKFNWYVDGVEVHNAKTKPREEQYNSTYRVVSVLTVLHQDWLNGKEYKCKVSNKALPAPIEKTISKAKGQPREPQVYTLPPSRDELTKNQVSLTCLVKGFYPSDIAVEWESNGQPENNYKTTPPVLDSDGSFFLYSKLTVDKSRWQQGNVFSCSVMHEALHNHYTQKSLSLSPGGRPGSGRPGSEVQLVESGGGLVQPGGSLRLSCAASGSSFSPYAMGWYRQAPGKQRELVSATSEGGFTLYADSVKGRFTISRDNSKNTVYLQMNSLRAEDTAVYYCYMHWRGSDPENYWGQGTQVTVSS

SEQ ID NO: 23 - protein, 486 aa, synthetic construct
EVQLLESGGGLVQPGGSLRLSCAASGFALDYYAIGWFRQAPGKGLEGVSCISSGEGSTYYADSVKGRFTISRDNSKNTVYLQMNSLRAEDTAVYYCATDSRGDDVACEGLRRNEYDYWGQGTLVTVSSGGGGGGGGGGSDTGRPFVEMYSEIPEIIHMTEGRELVIPCRVTSPNITVTLKKFPLDTLIPDGKRIIWDSRKGFIISNATYKEIGLLTCEATVNGHLYKTNYLTHRQTNTIIDVVLSPSHGIELSVGEKLVLNCTARTELNVGIDFNWEYPSSKHQHKKLVNRDLKTQSGSEMKKFLSTLTIDGVTRSDQGLYTCAASSGLMTKKNSTFVRVHEKEPKSSPPCPPCPAPCGGGGGGGGGGEVQLVESGGGLVQPGGSLRLSCAASGSSFSPYAMGWYRQAPGKQRELVSATSEGGFTLYADSVKGRFTISRDNSKNTVYLQMNSLRAEDTAVYYCYMHWRGSDPENYWGQGTQVTVSS

SEQ ID NO: 24 - protein, 485 aa, synthetic construct
EVQLLESGGGLVQPGGSLRLSCAASGFALDYYAIGWFRQAPGKGLEGVSCISSGEGSTYYADSVKGRFTISRDNSKNTVYLQMNSLRAEDTAVYYCATDSRGDDVACEGLRRNEYDYWGQGTLVTVSSGGGGGGGGGGSDTGRPFVEMYSEIPEIIHMTEGRELVIPCRVTSPNITVTLKKFPLDTLIPDGKRIIWDSRKGFIISNATYKEIGLLTCEATVNGHLYKTNYLTHRQTNTIIDVVLSPSHGIELSVGEKLVLNCTARTELNVGIDFNWEYPSSKHQHKKLVNRDLKTQSGSEMKKFLSTLTIDGVTRSDQGLYTCAASSGLMTKKNSTFVRVHEKESKYGPPCPPCPPCGGGGGGGGGGEVQLVESGGGLVQPGGSLRLSCAASGSSFSPYAMGWYRQAPGKQRELVSATSEGGFTLYADSVKGRFTISRDNSKNTVYLQMNSLRAEDTAVYYCYMHWRGSDPENYWGQGTQVTVSS

SEQ ID NO: 25 - protein, 483 aa, synthetic construct
EVQLLESGGGLVQPGGSLRLSCAASGFALDYYAIGWFRQAPGKGLEGVSCISSGEGSTYYADSVKGRFTISRDNSKNTVYLQMNSLRAEDTAVYYCATDSRGDDVACEGLRRNEYDYWGQGTLVTVSSGGGGGGGGGGSDTGRPFVEMYSEIPEIIHMTEGRELVIPCRVTSPNITVTLKKFPLDTLIPDGKRIIWDSRKGFIISNATYKEIGLLTCEATVNGHLYKTNYLTHRQTNTIIDVVLSPSHGIELSVGEKLVLNCTARTELNVGIDFNWEYPSSKHQHKKLVNRDLKTQSGSEMKKFLSTLTIDGVTRSDQGLYTCAASSGLMTKKNSTFVRVHEKEKTHTCPPCPPCGGGGGGGGGGEVQLVESGGGLVQPGGSLRLSCAASGSSFSPYAMGWYRQAPGKQRELVSATSEGGFTLYADSVKGRFTISRDNSKNTVYLQMNSLRAEDTAVYYCYMHWRGSDPENYWGQGTQVTVSS

SEQ ID NO: 26 - protein, 483 aa, synthetic construct
EVQLLESGGGLVQPGGSLRLSCAASGFALDYYAIGWFRQAPGKGLEGVSCISSGEGSTYYADSVKGRFTISRDNSKNTVYLQMNSLRAEDTAVYYCATDSRGDDVACEGLRRNEYDYWGQGTLVTVSSGGGGGGGGGGSDTGRPFVEMYSEIPEIIHMTEGRELVIPCRVTSPNITVTLKKFPLDTLIPDGKRIIWDSRKGFIISNATYKEIGLLTCEATVNGHLYKTNYLTHRQTNTIIDVVLSPSHGIELSVGEKLVLNCTARTELNVGIDFNWEYPSSKHQHKKLVNRDLKTQSGSEMKKFLSTLTIDGVTRSDQGLYTCAASSGLMTKKNSTFVRVHEKDTTHTCPPCPPCGGGGGGGGGGEVQLVESGGGLVQPGGSLRLSCAASGSSFSPYAMGWYRQAPGKQRELVSATSEGGFTLYADSVKGRFTISRDNSKNTVYLQMNSLRAEDTAVYYCYMHWRGSDPENYWGQGTQVTVSS

SEQ ID NO: 27 - protein, 486 aa, synthetic construct
EVQLLESGGGLVQPGGSLRLSCAASGFALDYYAIGWFRQAPGKGLEGVSCISSGEGSTYYADSVKGRFTISRDNSKNTVYLQMNSLRAEDTAVYYCATDSRGDDVACEGLRRNEYDYWGQGTLVTVSSGGGGGGGGGGSDTGRPFVEMYSEIPEIIHMTEGRELVIPCRVTSPNITVTLKKFPLDTLIPDGKRIIWDSRKGFIISNATYKEIGLLTCEATVNGHLYKTNYLTHRQTNTIIDVVLSPSHGIELSVGEKLVLNCTARTELNVGIDFNWEYPSSKHQHKKLVNRDLKTQSGSEMKKFLSTLTIDGVTRSDQGLYTCAASSGLMTKKNSTFVRVHEKEPKSCDTPPPCPPCPGGGGGGGGGGEVQLVESGGGLVQPGGSLRLSCAASGSSFSPYAMGWYRQAPGKQRELVSATSEGGFTLYADSVKGRFTISRDNSKNTVYLQMNSLRAEDTAVYYCYMHWRGSDPENYWGQGTQVTVSS

SEQ ID NO: 28 - protein, 488 aa, synthetic construct
EVQLLESGGGLVQPGGSLRLSCAASGFALDYYAIGWFRQAPGKGLEGVSCISSGEGSTYYADSVKGRFTISRDNSKNTVYLQMNSLRAEDTAVYYCATDSRGDDVACEGLRRNEYDYWGQGTLVTVSSGGGGGGGGGGSDTGRPFVEMYSEIPEIIHMTEGRELVIPCRVTSPNITVTLKKFPLDTLIPDGKRIIWDSRKGFIISNATYKEIGLLTCEATVNGHLYKTNYLTHRQTNTIIDVVLSPSHGIELSVGEKLVLNCTARTELNVGIDFNWEYPSSKHQHKKLVNRDLKTQSGSEMKKFLSTLTIDGVTRSDQGLYTCAASSGLMTKKNSTFVRVHEKEPKSSDTPPPCPPCPPCGGGGGGGGGGEVQLVESGGGLVQPGGSLRLSCAASGSSFSPYAMGWYRQAPGKQRELVSATSEGGFTLYADSVKGRFTISRDNSKNTVYLQMNSLRAEDTAVYYCYMHWRGSDPENYWGQGTQVTVSS

SEQ ID NO: 29 - protein, 486 aa, synthetic construct
SDTGRPFVEMYSEIPEIIHMTEGRELVIPCRVTSPNITVTLKKFPLDTLIPDGKRIIWDSRKGFIISNATYKEIGLLTCEATVNGHLYKTNYLTHRQTNTIIDVVLSPSHGIELSVGEKLVLNCTARTELNVGIDFNWEYPSSKHQHKKLVNRDLKTQSGSEMKKFLSTLTIDGVTRSDQGLYTCAASSGLMTKKNSTFVRVHEKEPKSSPPCPPCPAPCGGGGGGGGGGEVQLLESGGGLVQPGGSLRLSCAASGFALDYYAIGWFRQAPGKGLEGVSCISSGEGSTYYADSVKGRFTISRDNSKNTVYLQMNSLRAEDTAVYYCATDSRGDDVACEGLRRNEYDYWGQGTLVTVSSGGGGGGGGGGEVQLVESGGGLVQPGGSLRLSCAASGSSFSPYAMGWYRQAPGKQRELVSATSEGGFTLYADSVKGRFTISRDNSKNTVYLQMNSLRAEDTAVYYCYMHWRGSDPENYWGQGTQVTVSS

SEQ ID NO: 30 - protein, 485 aa, synthetic construct
SDTGRPFVEMYSEIPEIIHMTEGRELVIPCRVTSPNITVTLKKFPLDTLIPDGKRIIWDSRKGFIISNATYKEIGLLTCEATVNGHLYKTNYLTHRQTNTIIDVVLSPSHGIELSVGEKLVLNCTARTELNVGIDFNWEYPSSKHQHKKLVNRDLKTQSGSEMKKFLSTLTIDGVTRSDQGLYTCAASSGLMTKKNSTFVRVHEKESKYGPPCPPCPPCGGGGGGGGGGEVQLLESGGGLVQPGGSLRLSCAASGFALDYYAIGWFRQAPGKGLEGVSCISSGEGSTYYADSVKGRFTISRDNSKNTVYLQMNSLRAEDTAVYYCATDSRGDDVACEGLRRNEYDYWGQGTLVTVSSGGGGGGGGGGEVQLVESGGGLVQPGGSLRLSCAASGSSFSPYAMGWYRQAPGKQRELVSATSEGGFTLYADSVKGRFTISRDNSKNTVYLQMNSLRAEDTAVYYCYMHWRGSDPENYWGQGTQVTVSS

SEQ ID NO: 31 - protein, 483 aa, synthetic construct
SDTGRPFVEMYSEIPEIIHMTEGRELVIPCRVTSPNITVTLKKFPLDTLIPDGKRIIWDSRKGFIISNATYKEIGLLTCEATVNGHLYKTNYLTHRQTNTIIDVVLSPSHGIELSVGEKLVLNCTARTELNVGIDFNWEYPSSKHQHKKLVNRDLKTQSGSEMKKFLSTLTIDGVTRSDQGLYTCAASSGLMTKKNSTFVRVHEKEKTHTCPPCPPCGGGGGGGGGGEVQLLESGGGLVQPGGSLRLSCAASGFALDYYAIGWFRQAPGKGLEGVSCISSGEGSTYYADSVKGRFTISRDNSKNTVYLQMNSLRAEDTAVYYCATDSRGDDVACEGLRRNEYDYWGQGTLVTVSSGGGGGGGGGGEVQLVESGGGLVQPGGSLRLSCAASGSSFSPYAMGWYRQAPGKQRELVSATSEGGFTLYADSVKGRFTISRDNSKNTVYLQMNSLRAEDTAVYYCYMHWRGSDPENYWGQGTQVTVSS

SEQ ID NO: 32 - protein, 487 aa, synthetic construct
SDTGRPFVEMYSEIPEIIHMTEGRELVIPCRVTSPNITVTLKKFPLDTLIPDGKRIIWDSRKGFIISNATYKEIGLLTCEATVNGHLYKTNYLTHRQTNTIIDVVLSPSHGIELSVGEKLVLNCTARTELNVGIDFNWEYPSSKHQHKKLVNRDLKTQSGSEMKKFLSTLTIDGVTRSDQGLYTCAASSGLMTKKNSTFVRVHEKDKTHTCPPCPAPELLGGRPGSGRPGSEVQLLESGGGLVQPGGSLRLSCAASGFALDYYAIGWFRQAPGKGLEGVSCISSGEGSTYYADSVKGRFTISRDNSKNTVYLQMNSLRAEDTAVYYCATDSRGDDVACEGLRRNEYDYWGQGTLVTVSSGRPGSGRPGSEVQLVESGGGLVQPGGSLRLSCAASGSSFSPYAMGWYRQAPGKQRELVSATSEGGFTLYADSVKGRFTISRDNSKNTVYLQMNSLRAEDTAVYYCYMHWRGSDPENYWGQGTQVTVSS

SEQ ID NO: 33 - protein, 483 aa, synthetic construct
EVQLLESGGGLVQPGGSLRLSCAASGFALDYYAIGWFRQAPGKGLEGVSCISSGEGSTYYADSVKGRFTISRDNSKNTVYLQMNSLRAEDTAVYYCATDSRGDDVACEGLRRNEYDYWGQGTLVTVSSGGGGGGGGGGSDTGRPFVEMYSEIPEIIHMTEGRELVIPCRVTSPNITVTLKKFPLDTLIPDGKRIIWDSRKGFIISNATYKEIGLLTCEATVNGHLYKTNYLTHRQTNTIIDVVLSPSHGIELSVGEKLVLNCTARTELNVGIDFNWEYPSSKHQHKKLVNRDLKTQSGSEMKKFLSTLTIDGVTRSDQGLYTCAASSGLMTKKNSTFVRVHEKGGGGGGGGGGEVQLVESGGGLVQPGGSLRLSCAASGSSFSPYAMGWYRQAPGKQRELVSATSEGGFTLYADSVKGRFTISRDNSKNTVYLQMNSLRAEDTAVYYCYMHWRGSDPENYWGQGTQVTVSSDKTHTCPPCPPC

SEQ ID NO: 34 - protein, 483 aa, synthetic construct
EVQLLESGGGLVQPGGSLRLSCAASGFALDYYAIGWFRQAPGKGLEGVSCISSGEGSTYYADSVKGRFTISRDNSKNTVYLQMNSLRAEDTAVYYCATDSRGDDVACEGLRRNEYDYWGQGTLVTVSSGRPGSGRPGSSDTGRPFVEMYSEIPEIIHMTEGRELVIPCRVTSPNITVTLKKFPLDTLIPDGKRIIWDSRKGFIISNATYKEIGLLTCEATVNGHLYKTNYLTHRQTNTIIDVVLSPSHGIELSVGEKLVLNCTARTELNVGIDFNWEYPSSKHQHKKLVNRDLKTQSGSEMKKFLSTLTIDGVTRSDQGLYTCAASSGLMTKKNSTFVRVHEKGRPGSGRPGSEVQLVESGGGLVQPGGSLRLSCAASGSSFSPYAMGWYRQAPGKQRELVSATSEGGFTLYADSVKGRFTISRDNSKNTVYLQMNSLRAEDTAVYYCYMHWRGSDPENYWGQGTQVTVSSDKTHTCPPCPPC

SEQ ID NO: 35 - protein, 226 aa, synthetic construct
DKTHTCPPCPAPELLGGPSVFLFPPKPKDTLMISRTPEVTCVVVDVSHEDPEVKFNWYVDGVEVHNAKTKPREEQYNSTYRVVSVLTVLHQDWLNGKEYKCKVSNKALPAPIEKTISKAKGQPREPQVYTLPPSRDELTKNQVSLTCLVKGFYPSDIAVEWESNGQPENNYKTTPPVLDSDGSFFLYSKLTVDKSRWQQGNVFSCSVMHEALHNHYTQKSLSLSPG

SEQ ID NO: 36 - protein, 431 aa, synthetic construct
SDTGRPFVEMYSEIPEIIHMTEGRELVIPCRVTSPNITVTLKKFPLDTLIPDGKRIIWDSRKGFIISNATYKEIGLLTCEATVNGHLYKTNYLTHRQTNTIIDVVLSPSHGIELSVGEKLVLNCTARTELNVGIDFNWEYPSSKHQHKKLVNRDLKTQSGSEMKKFLSTLTIDGVTRSDQGLYTCAASSGLMTKKNSTFVRVHEKDKTHTCPPCPAPELLGGPSVFLFPPKPKDTLMISRTPEVTCVVVDVSHEDPEVKFNWYVDGVEVHNAKTKPREEQYNSTYRVVSVLTVLHQDWLNGKEYKCKVSNKALPAPIEKTISKAKGQPREPQVYTLPPSRDELTKNQVSLTCLVKGFYPSDIAVEWESNGQPENNYKTTPPVLDSDGSFFLYSKLTVDKSRWQQGNVFSCSVMHEALHNHYTQKSLSLSPG

SEQ ID NO: 37 - protein, 453 aa, synthetic construct
EVQLVESGGGLVQPGGSLRLSCAASGYDFTHYGMNWVRQAPGKGLEWVGWINTYTGEPTYAADFKRRFTFSLDTSKSTAYLQMNSLRAEDTAVYYCAKYPYYYGTSHWYFDVWGQGTLVTVSSASTKGPSVFPLAPSSKSTSGGTAALGCLVKDYFPEPVTVSWNSGALTSGVHTFPAVLQSSGLYSLSSVVTVPSSSLGTQTYICNVNHKPSNTKVDKKVEPKSCDKTHTCPPCPAPEAAGGPSVFLFPPKPKDTLMASRTPEVTCVVVDVSHEDPEVKFNWYVDGVEVHNAKTKPREEQYNSTYRVVSVLTVLAQDWLNGKEYKCKVSNKALGAPIEKTISKAKGQPREPQVYTLPPCRDELTKNQVSLWCLVKGFYPSDIAVEWESNGQPENNYKTTPPVLDSDGSFFLYSKLTVDKSRWQQGNVFSCSVMHEALHNAYTQKSLSLSPGK

SEQ ID NO: 38 - protein, 463 aa, synthetic construct
QVQLVQSGAEVKKPGASVKVSCKASGYTFTGYYMHWVRQAPGQGLEWMGWINPNSGGTNYAQKFQGRVTMTRDTSISTAYMELSRLRSDDTAVYYCARSPNPYYYDSSGYYYPGAFDIWGQGTMVTVSSASVAAPSVFIFPPSDEQLKSGTASVVCLLNNFYPREAKVQWKVDNALQSGNSQESVTEQDSKDSTYSLSSTLTLSKADYEKHKVYACEVTHQGLSSPVTKSFNRGECDKTHTCPPCPAPEAAGGPSVFLFPPKPKDTLMASRTPEVTCVVVDVSHEDPEVKFNWYVDGVEVHNAKTKPREEQYNSTYRVVSVLTVLAQDWLNGKEYKCKVSNKALGAPIEKTISKAKGQPREPQVCTLPPSRDELTKNQVSLSCAVKGFYPSDIAVEWESNGQPENNYKTTPPVLDSDGSFFLVSKLTVDKSRWQQGNVFSCSVMHEALHNAYTQKSLSLSPGK

SEQ ID NO: 39 - protein, 214 aa, synthetic construct
DIQLTQSPSSLSASVGDRVTITCSASQDISNYLNWYQQKPGKAPKVLIYFTSSLHSGVPSRFSGSGSGTDFTLTISSLQPEDFATYYCQQYSTVPWTFGQGTKVEIKRTVAAPSVFIFPPSDEQLKSGTASVVCLLNNFYPREAKVQWKVDNALQSGNSQESVTEQDSKDSTYSLSSTLTLSKADYEKHKVYACEVTHQGLSSPVTKSFNRGEC

SEQ ID NO: 40 - protein, 213 aa, synthetic construct
SYVLTQPPSVSVAPGQTARITCGGNNIGSKSVHWYQQKPGQAPVLVVYDDSDRPSGIPERFSGSNSGNTATLTISRVEAGDEADYYCQVWDSSSDHWVFGGGTKLTVLSSASTKGPSVFPLAPSSKSTSGGTAALGCLVKDYFPEPVTVSWNSGALTSGVHTFPAVLQSSGLYSLSSVVTVPSSSLGTQTYICNVNHKPSNTKVDKKVEPKSC

SEQ ID NO: 41 - protein, 537 aa, synthetic construct
YSMTPPTLNITEESHVIDTGDSLSISCRGQHPLEWAWPGAQEAPATGDKDSEDTGVVRDCEGTDARPYCKVLLLHEVHAQDTGSYVCYYKYIKARIEGTTAASSYVFVRDFEQPFINKPDTLLVNRKDAMWVPCLVSIPGLNVTLRSQSSVLWPDGQEVVWDDRRGMLVSTPLLHDALYLQCETTWGDQDFLSNPFLVHITGNELYDIQLLPRKSLELLVGEKLVLNCTVWAEFNSGVTFDWDYPGKQAERGKWVPERRSQQTHTELSSILTIHNVSQHDLGSYVCKANNGIQRFRESTEVIVHEEPKSCDKTHTCPPCPAPELLGGPSVFLFPPKPKDTLMISRTPEVTCVVVDVSHEDPEVKFNWYVDGVEVHNAKTKPREEQYNSTYRVVSVLTVLHQDWLNGKEYKCKVSNKALPAPIEKTISKAKGQPREPQVYTLPPSRDELTKNQVSLTCLVKGFYPSDIAVEWESNGQPENNYKTTPPVLDSDGSFFLYSKLTVDKSRWQQGNVFSCSVMHEALHNHYTQKSLSLSPGK

SEQ ID NO: 42 - protein, 393 aa, synthetic construct
DIQLTQSPSSLSASVGDRVTITCSASQDISNYLNWYQQKPGKAPKVLIYFTSSLHSGVPSRFSGSGSGTDFTLTISSLQPEDFATYYCQQYSTVPWTFGCGTKVEIKGGGGSGGGGSGGGGSGGGGSEVQLVESGGGLVQPGGSLRLSCAASGYDFTHYGMNWVRQAPGKCLEWVGWINTYTGEPTYAADFKRRFTFSLDTSKSTAYLQMNSLRAEDTAVYYCAKYPYYYGTSHWYFDVWGQGTLVTVSSGGGGSGGGGSGGGGSEVQLLESGGGLVQPGGSLRLSCAASGFALDYYAIGWFRQAPGKGLEGVSCISSGEGSTYYADSVKGRFTISRDNSKNTVYLQMNSLRAEDTAVYYCATDSRGDDVACEGLRRNEYDYWGQGTLVTVSS

SEQ ID NO: 43 - protein, 574 aa, synthetic construct
SDTGRPFVEMYSEIPEIIHMTEGRELVIPCRVTSPNITVTLKKFPLDTLIPDGKRIIWDSRKGFIISNATYKEIGLLTCEATVNGHLYKTNYLTHRQTNTIIDVVLSPSHGIELSVGEKLVLNCTARTELNVGIDFNWEYPSSKHQHKKLVNRDLKTQSGSEMKKFLSTLTIDGVTRSDQGLYTCAASSGLMTKKNSTFVRVHEKDKTHTCPPCPAPELLGGPSVFLFPPKPKDTLMISRTPEVTCVVVDVSHEDPEVKFNWYVDGVEVHNAKTKPREEQYNSTYRVVSVLTVLHQDWLNGKEYKCKVSNKALPAPIEKTISKAKGQPREPQVYTLPPSRDELTKNQVSLTCLVKGFYPSDIAVEWESNGQPENNYKTTPPVLDSDGSFFLYSKLTVDKSRWQQGNVFSCSVMHEALHNHYTQKSLSLSPGGGGGSGGGGSGGGGSEVQLLESGGGLVQPGGSLRLSCAASGFALDYYAIGWFRQAPGKGLEGVSCISSGEGSTYYADSVKGRFTISRDNSKNTVYLQMNSLRAEDTAVYYCATDSRGDDVACEGLRRNEYDYWGQGTLVTVSS

SEQ ID NO: 44 - protein, 564 aa, synthetic construct
SDTGRPFVEMYSEIPEIIHMTEGRELVIPCRVTSPNITVTLKKFPLDTLIPDGKRIIWDSRKGFIISNATYKEIGLLTCEATVNGHLYKTNYLTHRQTNTIIDVVLSPSHGIELSVGEKLVLNCTARTELNVGIDFNWEYPSSKHQHKKLVNRDLKTQSGSEMKKFLSTLTIDGVTRSDQGLYTCAASSGLMTKKNSTFVRVHEKDKTHTCPPCPAPELLGGPSVFLFPPKPKDTLMISRTPEVTCVVVDVSHEDPEVKFNWYVDGVEVHNAKTKPREEQYNSTYRVVSVLTVLHQDWLNGKEYKCKVSNKALPAPIEKTISKAKGQPREPQVYTLPPSRDELTKNQVSLTCLVKGFYPSDIAVEWESNGQPENNYKTTPPVLDSDGSFFLYSKLTVDKSRWQQGNVFSCSVMHEALHNHYTQKSLSLSPGGGGGSGGGGSGGGGSEVQLVESGGGLVQPGGSLRLSCAASGSSFSPYAMGWYRQAPGKQRELVSATSSGGFTLYADSVKGRFTISRDNSKNTVYLQMNSLRAEDTAVYYCYTYYREYDPEMYWGQGTQVTVSS

SEQ ID NO: 45 - protein, 18 aa, synthetic construct
EPKSSPPCPPCPAPCLLG

SEQ ID NO: 46 - protein, 16 aa, synthetic construct
DKTHTCPPCPAPCLLG

SEQ ID NO: 47 - protein, 106 aa, synthetic construct [sequence omitted]

SEQ ID NO: 48 - protein, 489 aa, synthetic construct
EVQLLESGGGLVQPGGSLRLSCAASGFALDYYAIGWFRQAPGKGLEGVSCISSGEGSTYYADSVKGRFTISRDNSKNTVYLQMNSLRAEDTAVYYCATDSRGDDVACEGLRRNEYDYWGQGTLVTVSSGGGGGGGGGGSDTGRPFVEMYSEIPEIIHMTEGRELVIPCRVTSPNITVTLKKFPLDTLIPDGKRIIWDSRKGFIISNATYKEIGLLTCEATVNGHLYKTNYLTHRQTNTIIDVVLSPSHGIELSVGEKLVLNCTARTELNVGIDFNWEYPSSKHQHKKLVNRDLKTQSGSEMKKFLSTLTIDGVTRSDQGLYTCAASSGLMTKKNSTFVRVHEKEPKSSPPCPPCPAPCLLGGGGGGGGGGGEVQLVESGGGLVQPGGSLRLSCAASGSSFSPYAMGWYRQAPGKQRELVSATSEGGFTLYADSVKGRFTISRDNSKNTVYLQMNSLRAEDTAVYYCYMHWRGSDPENYWGQGTQVTVSS

SEQ ID NO: 49 - protein, 593 aa, synthetic construct
EVQLLESGGGLVQPGGSLRLSCAASGFALDYYAIGWFRQAPGKGLEGVSCISSGEGSTYYADSVKGRFTISRDNSKNTVYLQMNSLRAEDTAVYYCATDSRGDDVACEGLRRNEYDYWGQGTLVTVSSGGGGGGGGGGSDTGRPFVEMYSEIPEIIHMTEGRELVIPCRVTSPNITVTLKKFPLDTLIPDGKRIIWDSRKGFIISNATYKEIGLLTCEATVNGHLYKTNYLTHRQTNTIIDVVLSPSHGIELSVGEKLVLNCTARTELNVGIDFNWEYPSSKHQHKKLVNRDLKTQSGSEMKKFLSTLTIDGVTRSDQGLYTCAASSGLMTKKNSTFVRVHEKDKTHTCPPCPAPELLGGQPREPQVYTLPPSRDELTKNQVSLTCLVKGFYPSDIAVEWESNGQPENNYKTTPPVLDSDGSFFLYSKLTVDKSRWQQGNVFSCSVMHEALHNHYTQKSLSLSPGGGGGGGGGGGEVQLVESGGGLVQPGGSLRLSCAASGSSFSPYAMGWYRQAPGKQRELVSATSEGGFTLYADSVKGRFTISRDNSKNTVYLQMNSLRAEDTAVYYCYMHWRGSDPENYWGQGTQVTVSS

SEQ ID NO: 50 - protein, 487 aa, synthetic construct
EVQLLESGGGLVQPGGSLRLSCAASGFALDYYAIGWFRQAPGKGLEGVSCISSGEGSTYYADSVKGRFTISRDNSKNTVYLQMNSLRAEDTAVYYCATDSRGDDVACEGLRRNEYDYWGQGTLVTVSSGGGGGGGGGGSDTGRPFVEMYSEIPEIIHMTEGRELVIPCRVTSPNITVTLKKFPLDTLIPDGKRIIWDSRKGFIISNATYKEIGLLTCEATVNGHLYKTNYLTHRQTNTIIDVVLSPSHGIELSVGEKLVLNCTARTELNVGIDFNWEYPSSKHQHKKLVNRDLKTQSGSEMKKFLSTLTIDGVTRSDQGLYTCAASSGLMTKKNSTFVRVHEKDKTHTCPPCPAPCLLGGGGGGGGGGGEVQLVESGGGLVQPGGSLRLSCAASGSSFSPYAMGWYRQAPGKQRELVSATSEGGFTLYADSVKGRFTISRDNSKNTVYLQMNSLRAEDTAVYYCYMHWRGSDPENYWGQGTQVTVSS

SEQ ID NO: 51 - protein, 15 aa, synthetic construct
DKTHTCPPCPPCPPC

SEQ ID NO: 52 - protein, 11 aa, synthetic construct
ERKCCVECPPC

SEQ ID NO: 53 - protein, 15 aa, synthetic construct
EPKSCDTPPPCPRCP

SEQ ID NO: 54 - protein, 9 aa, synthetic construct
EPCCCPKCP

SEQ ID NO: 55 - protein, 5 aa, synthetic construct
  REPEAT 1..5: note = repeat n times, wherein n is an integer equal to or greater than 1
GGGGS

SEQ ID NO: 56 - protein, 7 aa, synthetic construct
  REPEAT 3..7: note = repeat n times, wherein n is an integer equal to or greater than 1
TSGGGGS

SEQ ID NO: 57 - protein, 6 aa, synthetic construct
  REPEAT 2..6: note = repeat n time, wherein n is an integer equal to or greater than 1
GGGGGS

SEQ ID NO: 58 - protein, 5 aa, synthetic construct
  REPEAT 1..5: note = repeat n time, wherein n is an integer equal to or greater than 2
GGGGG

SEQ ID NO: 59 - protein, 5 aa, synthetic construct
  REPEAT 1..5: note = repeat n times, wherein n is an integer equal to or greater than 2
GRPGS

SEQ ID NO: 60 - protein, 4 aa, synthetic construct
CPPC

SEQ ID NO: 61 - protein, 7 aa, synthetic construct
CPPCPPC

SEQ ID NO: 62 - protein, 10 aa, synthetic construct
GGGGSGGGGS

SEQ ID NO: 63 - protein, 15 aa, synthetic construct
GGGGSGGGGSGGGGS

SEQ ID NO: 64 - protein, 28 aa, synthetic construct
EPKSSPPCPPCPAPCLLGGGGGGGGGGG

SEQ ID NO: 65 - protein, 122 aa, synthetic construct
DKTHTCPPCPAPELLGGQPREPQVYTLPPSRDELTKNQVSLTCLVKGFYPSDIAVEWESNGQPENNYKTTPPVLDSDGSFFLYSKLTVDKSRWQQGNVFSCSVMHEALHNHYTQKSLSLSPG

SEQ ID NO: 66 - protein, 26 aa, synthetic construct
EPKSSPPCPPCPAPCGGGGGGGGGGG

SEQ ID NO: 67 - protein, 27 aa, synthetic construct
DKTHTCPPCPAPCLLGGGGGGGGGGGG

SEQ ID NO: 68 - protein, 23 aa, synthetic construct
DTTHTCPPCPPCGGGGGGGGGGG

SEQ ID NO: 69 - protein, 26 aa, synthetic construct
EPKSCDTPPPCPPCPGGGGGGGGGGG

SEQ ID NO: 70 - protein, 28 aa, synthetic construct
EPKSSDTPPPCPPCPPCGGGGGGGGGGG